European Patent Specification EP 3 472 165 B1, published September 6, 2023. Title: N-(substituted-phenyl)-sulfonamide derivatives as kinase inhibitors. Applicant: Nerviano Medical Sciences S.r.l. The sequence listing filed with the application follows.

SEQUENCE LISTING (1 sequence)

SEQ ID NO: 1 - protein, 15 aa, Artificial
  peptide substrate
LLSELSRRRIRSINK